European Patent Specification EP 3 412 300 B1, published July 29, 2026. Title: THERAPEUTIC AGENTS COMPRISING ELASTIN-LIKE PEPTIDES. Applicant: Chilkoti, Ashutosh. The sequence listing filed with the application follows.

SEQUENCE LISTING (59 sequences)

SEQ ID NO: 1 - protein, 4 aa, Artificial Sequence
  ELP component sequence
VPGG

SEQ ID NO: 2 - protein, 4 aa, Artificial Sequence
  ELP component sequence
IPGG

SEQ ID NO: 3 - protein, 5 aa, Artificial Sequence
  ELP component sequence
  misc_feature (4)..(4): Xaa can be any naturally occurring or non-natural amino acid
VPGXG

SEQ ID NO: 4 - protein, 5 aa, Artificial Sequence
  ELP component sequence
AVGVP

SEQ ID NO: 5 - protein, 5 aa, Artificial Sequence
  ELP component sequence
  misc_feature (4)..(4): Xaa can be any naturally occurring or non-natural amino acid
IPGXG

SEQ ID NO: 6 - protein, 5 aa, Artificial Sequence
  ELP component sequence
IPGVG

SEQ ID NO: 7 - protein, 5 aa, Artificial Sequence
  ELP component sequence
  misc_feature (4)..(4): Xaa can be any naturally occurring or non-natural amino acid
LPGXG

SEQ ID NO: 8 - protein, 5 aa, Artificial Sequence
  ELP component sequence
LPGVG

SEQ ID NO: 9 - protein, 6 aa, Artificial Sequence
  ELP component sequence
VAPGVG

SEQ ID NO: 10 - protein, 8 aa, Artificial Sequence
  ELP component sequence
GVGVPGVG

SEQ ID NO: 11 - protein, 9 aa, Artificial Sequence
  ELP component sequence
VPGFGVGAG

SEQ ID NO: 12 - protein, 9 aa, Artificial Sequence
  ELP component sequence
VPGVGVPGG

SEQ ID NO: 13 - protein, 30 aa, Homo sapiens
HAEGTFTSDVSSYLEGQAAKEFIAWLVKGR

SEQ ID NO: 14 - protein, 38 aa, Homo sapiens
HGEGTFTSDLSKQMEEEAVRLFEWLKNGGPSSGAPPPS

SEQ ID NO: 15 - protein, 21 aa, Homo sapiens
GIVEQCCASVCSLYQLENYCN

SEQ ID NO: 16 - protein, 30 aa, Homo sapiens
FVNQHLCGSHLVEALYLVCGERGFFYTPKA

SEQ ID NO: 17 - protein, 30 aa, Homo sapiens
HGEGTFTSDVSSYLEGQAAKEFIAWLVKGR

SEQ ID NO: 18 - protein, 44 aa, Unknown
  GLP-1 receptor agonist
HGEGTFTSDLSKQMEEEAVRLFIEWLKNGGPSSGAPPSKKKKKK

SEQ ID NO: 19 - protein, 31 aa, Unknown
  GLP-1 receptor agonist
HVEGTFTSDVSSYLEEQAAKEFIAWLIKGRG

SEQ ID NO: 20 - protein, 12 aa, Artificial Sequence
  Peptide linker sequence
KDDNPNLPRLVR

SEQ ID NO: 21 - protein, 12 aa, Artificial Sequence
  Peptide linker sequence
GAGSSSRRAPQT

SEQ ID NO: 22 - protein, 8 aa, Artificial Sequence
  Non-cleavable spacer sequence
  MISC_FEATURE (2)..(4): Gly residue is optional
  MISC_FEATURE (6)..(8): Ser residue is optional
GGGGSSSS

SEQ ID NO: 23 - DNA, 300 bp, Artificial Sequence
  Exendin-4/ELP sequence
aattaatacgactcactataggggaattgtgagcggataacaattcccctctagaaataattttgtttaactttaagaaggagatatacatatgcatggcgaaggcacctttaccagcgatctgagcaaacagatggaagaagaagcggtgcgcctgtttattgaatggctgaaaaacggcggcccgagcagcggcgcgccgccgccgagcctcgagggcatgggtgggccgggcgtgggtgttccgggcgtgggtgttccgggtggcggtgtgccgggcgcaggtgttcctggtgtagg

SEQ ID NO: 24 - protein, 69 aa, Artificial Sequence
  Exendin-4/ELP sequence
MHGEGTFTSDLSKQMEEEAVRLFIEWLKNGGPSSGAPPPSLEGMGGPGVGVPGVGVPGGGVPGAGVPGV

SEQ ID NO: 25 - DNA, 140 bp, Artificial Sequence
  Exendin-4/ELP sequence with N-terminal Tev cleavage site
tatggaaaacctgtatttccaacatggcgaaggcacctttaccagcgatctgagcaaacagatggaagaagaagcggtgcgcctgtttattgaatggctgaaaaacggcggcccgagcagcggcgcgccgccgccgagcc

SEQ ID NO: 26 - protein, 46 aa, Artificial Sequence
  Exendin-4/ELP sequence with N-terminal Tev cleavage site
MENLYFQHGEGTFTSDLSKQMEEEAVRLFIEWLKNGGPSSGAPPPS

SEQ ID NO: 27 - DNA, 155 bp, Artificial Sequence
  Exendin-4/ELP sequence with N-terminal Tev cleavage site and additional N-terminal sequence
tatggatatcccaacgaccgaaaacctgtatttccaacatggcgaaggcacctttaccagcgatctgagcaaacagatggaagaagaagcggtgcgcctgtttattgaatggctgaaaaacggcggcccgagcagcggcgcgccgccgccgagcc

SEQ ID NO: 28 - protein, 51 aa, Artificial Sequence
  Exendin-4/ELP sequence with N-terminal Tev cleavage site and additional N-terminal sequence
MDIPTTENLYFQHGEGTFTSDLSKQMEEEAVRLFIEWLKNGGPSSGAPPPS

SEQ ID NO: 29 - DNA, 176 bp, Artificial Sequence
  Exendin-4/ELP sequence with DsbA leader sequence
tatgaaaaagatttggctggcgctggctggtttagttttagcgtttagcgcatcggcgcatggcgaaggcacctttaccagcgatctgagcaaacagatggaagaagaagcggtgcgcctgtttattgaatggctgaaaaacggcggcccgagcagcggcgcgccgccgccgagcc

SEQ ID NO: 30 - protein, 58 aa, Artificial Sequence
  Exendin-4/ELP sequence with DsbA leader sequence
MKKIWLALAGLVLAFSASAHGEGTFTSDLSKQMEEEAVRLFIEWLKNGGPSSGAPPPS

SEQ ID NO: 31 - DNA, 400 bp, Artificial Sequence
  Insulin/ELP sequence
ctagaaataattttgtttaactttaagaaggagatatacatatgtttgtgaaccaacacctgtgcggctcacacctggtggaagctctctacctagtgtgcggggaacgaggcttcttctacacacccaagacccgccgggaggcagaggacctgcaggtggggcaggtggagctgggcgggggccctggtgcaggcagcctgcagcccttggccctggaggggtccctgcagaagcgtggcattgtggaacaatgctgtaccagcatctgctccctctaccagctggagaactactgcaacctcgagggcatgggtgggccgggcgtgggtgttccgggcgtgggtgttccgggtggcggtgtgccgggcgcaggtgttcctggtgtaggtgtgccggg

SEQ ID NO: 32 - protein, 119 aa, Artificial Sequence
  Insulin/ELP sequence
MFVNQHLCGSHLVEALYLVCGERGFFYTPKTRREAEDLQVGQVELGGGPGAGSLQPLALEGSLQKRGIVEQCCTSICSLYQLENYCNLEGMGGPGVGVPGVGVPGGGVPGAGVPGVGVP

SEQ ID NO: 33 - protein, 406 aa, Homo sapiens [sequence omitted]

SEQ ID NO: 34 - DNA, 1218 bp, Homo sapiens
gccaacgcgttcctggaggagctgcggccgggctccctggagagggagtgcaaggaggagcagtgctccttcgaggaggcccgggagatcttcaaggacgcggagaggacgaagctgttctggatttcttacagtgatggggaccagtgtgcctcaagtccatgccagaatgggggctcctgcaaggaccagctccagtcctatatctgcttctgcctccctgccttcgagggccggaactgtgagacgcacaaggatgaccagctgatctgtgtgaacgagaacggcggctgtgagcagtactgcagtgaccacacgggcaccaagcgctcctgtcggtgccacgaggggtactctctgctggcagacggggtgtcctgcacacccacagttgaatatccatgtggaaaaatacctattctagaaaaaagaaatgccagcaaaccccaaggccgaattgtggggggcaaggtgtgccccaaaggggagtgtccatggcaggtcctgttgttggtgaatggagctcagttgtgtggggggaccctgatcaacaccatctgggtggtctccgcggcccactgtttcgacaaaatcaagaactggaggaacctgatcgcggtgctgggcgagcacgacctcagcgagcacgacggggatgagcagagccggcgggtggcgcaggtcatcatccccagcacgtacgtcccgggcaccaccaaccacgacatcgcgctgctccgcctgcaccagcccgtggtcctcactgaccatgtggtgcccctctgcctgcccgaacggacgttctctgagaggacgctggccttcgtgcgcttctcattggtcagcggctggggccagctgctggaccgtggcgccacggccctggagctcatggtgctcaacgtgccccggctgatgacccaggactgcctgcagcagtcacggaaggtgggagactccccaaatatcacggagtacatgttctgtgccggctactcggatggcagcaaggactcctgcaagggggacagtggaggcccacatgccacccactaccggggcacgtggtacctgacgggcatcgtcagctggggccagggctgcgcaaccgtgggccactttggggtgtacaccagggtctcccagtacatcgagtggctgcaaaagctcatgcgctcagagccacgcccaggagtcctcctgcgagccccatttccc

SEQ ID NO: 35 - DNA, 33 bp, Homo sapiens
tatgcatggcgaaggcacctttaccagcgatct

SEQ ID NO: 36 - DNA, 62 bp, Homo sapiens
gagcaaacagatggaagaagaagcggtgcgcctgtttattgaatggctgaaaaacggcggcc

SEQ ID NO: 37 - DNA, 27 bp, Homo sapiens
cgagcagcggcgcgccgccgccgagcc

SEQ ID NO: 38 - DNA, 35 bp, Homo sapiens
tcgaggctcggcggcggcgcgccgctgctcgggcc

SEQ ID NO: 39 - DNA, 63 bp, Homo sapiens
gccgtttttcagccattcaataaacaggcgcaccgcttcttcttccatctgtttgctcagatc

SEQ ID NO: 40 - DNA, 26 bp, Homo sapiens
gctggtaaaggtgccttcgccatgca

SEQ ID NO: 41 - DNA, 51 bp, Artificial Sequence
  Primer for Exendin-4/ELP sequence with N-terminal Tev cleavage site
tatggaaaacctgtatttccaacatggcgaaggcacctttaccagcgatct

SEQ ID NO: 42 - DNA, 44 bp, Artificial Sequence
  Primer for Exendin-4/ELP sequence with N-terminal Tev cleavage site
gctggtaaaggtgccttcgccatgttggaaatacaggttttcca

SEQ ID NO: 43 - DNA, 66 bp, Artificial Sequence
  Primer for Exendin-4/ELP sequence with N-terminal Tev cleavage site and additional N-terminal sequence
tatggatatcccaacgaccgaaaacctgtatttccaacatggcgaaggcacctttaccagcgatct

SEQ ID NO: 44 - DNA, 59 bp, Artificial Sequence
  Primer for
gctggtaaaggtgccttcgccatgttggaaatacaggttttcggtcgttgggatatcca

SEQ ID NO: 45 - DNA, 87 bp, Artificial Sequence
  Primer for Exendin-4/ELP sequence with DsbA leader sequence
tatgaaaaagatttggctggcgctggctggtttagttttagcgtttagcgcatcggcgcatggcgaaggcacctttaccagcgatct

SEQ ID NO: 46 - DNA, 80 bp, Artificial Sequence
  Primer for Exendin-4/ELP sequence with DsbA leader sequence
gctggtaaaggtgccttcgccatgcgccgatgcgctaaacgctaaaactaaaccagccagcgccagccaaatctttttca

SEQ ID NO: 47 - DNA, 39 bp, Artificial Sequence
  Primer for Insulin/ELP sequence
gaaggagatatacatatgtttgtgaaccaacacctgtgc

SEQ ID NO: 48 - DNA, 30 bp, Artificial Sequence
  Primer for Insulin/ELP sequence
cccatgccctcgaggttgcagtagttctcc

SEQ ID NO: 49 - DNA, 27 bp, Homo sapiens
ctagctagcatggtctcccaggccctc

SEQ ID NO: 50 - DNA, 33 bp, Homo sapiens
tattcttgcggccgcgggaaatggggctcgcag

SEQ ID NO: 51 - DNA, 261 bp, Homo sapiens
atgtttgtgaaccaacacctgtgcggctcacacctggtggaagctctctacctagtgtgcggggaacgaggcttcttctacacacccaagacccgccgggaggcagaggacctgcaggtggggcaggtggagctgggcgggggccctggtgcaggcagcctgcagcccttggccctggaggggtccctgcagaagcgtggcattgtggaacaatgctgtaccagcatctgctccctctaccagctggagaactactgcaac

SEQ ID NO: 52 - protein, 87 aa, Homo sapiens
MFVNQHLCGSHLVEALYLVCGERGFFYTPKTRREAEDLQVGQVELGGGPGAGSLQPLALEGSLQKRGIVEQCCTSICSLYQLENYCN

SEQ ID NO: 53 - DNA, 1700 bp, Artificial Sequence
  pPB0868 DNA sequence
taatacgactcactataggggaattgtgagcggataacaattcccctctagaaataattttgtttaactttaagaaggagatatacatatggagaacctgtatttccaacatggcgaaggtacctttacaagcgatgttagttcatatctggagggccaggcggcaaaggaattcattgcgtggctggtgaaaggccgcggcctcgagggcatgggtgggccgggcgtgggtgttccgggcgtgggtgttccgggtggcggtgtgccgggcgcaggtgttcctggtgtaggtgtgccgggtgttggtgtgccgggtgttggtgtaccaggtggcggtgttccgggtgcaggcgttccgggtggcggtgtgccgggcgtgggtgttccgggcgtgggtgttccgggtggcggtgtgccgggcgcaggtgttcctggtgtaggtgtgccgggtgttggtgtgccgggtgttggtgtaccaggtggcggtgttccgggtgcaggcgttccgggtggcggtgtgccgggcgtgggtgttccgggcgtgggtgttccgggtggcggtgtgccgggcgcaggtgttcctggtgtaggtgtgccgggtgttggtgtgccgggtgttggtgtaccaggtggcggtgttccgggtgcaggcgttccgggtggcggtgtgccgggcgtgggtgttccgggcgtgggtgttccgggtggcggtgtgccgggcgcaggtgttcctggtgtaggtgtgccgggtgttggtgtgccgggtgttggtgtaccaggtggcggtgttccgggtgcaggcgttccgggtggcggtgtgccgggcgtgggtgttccgggcgtgggtgttccgggtggcggtgtgccgggcgcaggtgttcctggtgtaggtgtgccgggtgttggtgtgccgggtgttggtgtaccaggtggcggtgttccgggtgcaggcgttccgggtggcggtgtgccgggcgtgggtgttccgggcgtgggtgttccgggtggcggtgtgccgggcgcaggtgttcctggtgtaggtgtgccgggtgttggtgtgccgggtgttggtgtaccaggtggcggtgttccgggtgcaggcgttccgggtggcggtgtgccgggcgtgggtgttccgggcgtgggtgttccgggtggcggtgtgccgggcgcaggtgttcctggtgtaggtgtgccgggtgttggtgtgccgggtgttggtgtaccaggtggcggtgttccgggtgcaggcgttccgggtggcggtgtgccgggcgtgggtgttccgggcgtgggtgttccgggtggcggtgtgccgggcgcaggtgttcctggtgtaggtgtgccgggtgttggtgtgccgggtgttggtgtaccaggtggcggtgttccgggtgcaggcgttccgggtggcggtgtgccgggcgtgggtgttccgggcgtgggtgttccgggtggcggtgtgccgggcgcaggtgttcctggtgtaggtgtgccgggtgttggtgtgccgggtgttggtgtaccaggtggcggtgttccgggtgcaggcgttccgggtggcggtgtgccgggctggccgtgataagctagcatgactggtggacagcaaatgggtcggatccgaattcgagctccgtcgagcaccaccaccaccaccactgagatccggctgctaacaaagcccgaaaggaagctga

SEQ ID NO: 54 - protein, 498 aa, Artificial Sequence
  GLP-1(A8G,7-37)ELP1-90 amino acid sequence
MENLYFQHGEGTFTSDVSSYLEGQAAKEFIAWLVKGRGLEGMGGPGVGVPGVGVPGGGVPGAGVPGVGVPGVGVPGVGVPGGGVPGAGVPGGGVPGVGVPGVGVPGGGVPGAGVPGVGVPGVGVPGVGVPGGGVPGAGVPGGGVPGVGVPGVGVPGGGVPGAGVPGVGVPGVGVPGVGVPGGGVPGAGVPGGGVPGVGVPGVGVPGGGVPGAGVPGVGVPGVGVPGVGVPGGGVPGAGVPGGGVPGVGVPGVGVPGGGVPGAGVPGVGVPGVGVPGVGVPGGGVPGAGVPGGGVPGVGVPGVGVPGGGVPGAGVPGVGVPGVGVPGVGVPGGGVPGAGVPGGGVPGVGVPGVGVPGGGVPGAGVPGVGVPGVGVPGVGVPGGGVPGAGVPGGGVPGVGVPGVGVPGGGVPGAGVPGVGVPGVGVPGVGVPGGGVPGAGVPGGGVPGVGVPGVGVPGGGVPGAGVPGVGVPGVGVPGVGVPGGGVPGAGVPGGGVPGWP

SEQ ID NO: 55 - DNA, 2050 bp, Artificial Sequence
  pPB1022 DNA sequence
taatacgactcactataggggaattgtgagcggataacaattcccctctagaaataattttgtttaactttaagaaggagatatacatatggagaacctgtatttccaacatggcgaaggtacctttacaagcgatgttagttcatatctggagggccaggcggcaaaggaatttattgcgtggctggtgaaaggccgcggcgtgccgggcgtgggtgttccgggcgtgggtgttccgggtggcggtgtgccgggcgcaggtgttcctggtgtaggtgtgccgggtgttggtgtgccgggtgttggtgtaccaggtggcggtgttccgggtgcaggcgttccgggtggcggtgtgccgggcgtgggtgttccgggcgtgggtgttccgggtggcggtgtgccgggcgcaggtgttcctggtgtaggtgtgccgggtgttggtgtgccgggtgttggtgtaccaggtggcggtgttccgggtgcaggcgttccgggtggcggtgtgccgggcgtgggtgttccgggcgtgggtgttccgggtggcggtgtgccgggcgcaggtgttcctggtgtaggtgtgccgggtgttggtgtgccgggtgttggtgtaccaggtggcggtgttccgggtgcaggcgttccgggtggcggtgtgccgggcgtgggtgttccgggcgtgggtgttccgggtggcggtgtgccgggcgcaggtgttcctggtgtaggtgtgccgggtgttggtgtgccgggtgttggtgtaccaggtggcggtgttccgggtgcaggcgttccgggtggcggtgtgccgggcgtgggtgttccgggcgtgggtgttccgggtggcggtgtgccgggcgcaggtgttcctggtgtaggtgtgccgggtgttggtgtgccgggtgttggtgtaccaggtggcggtgttccgggtgcaggcgttccgggtggcggtgtgccgggcgtgggtgttccgggcgtgggtgttccgggtggcggtgtgccgggcgcaggtgttcctggtgtaggtgtgccgggtgttggtgtgccgggtgttggtgtaccaggtggcggtgttccgggtgcaggcgttccgggtggcggtgtgccgggcgtgggtgttccgggcgtgggtgttccgggtggcggtgtgccgggcgcaggtgttcctggtgtaggtgtgccgggtgttggtgtgccgggtgttggtgtaccaggtggcggtgttccgggtgcaggcgttccgggtggcggtgtgccgggcgtgggtgttccgggcgtgggtgttccgggtggcggtgtgccgggcgcaggtgttcctggtgtaggtgtgccgggtgttggtgtgccgggtgttggtgtaccaggtggcggtgttccgggtgcaggcgttccgggtggcggtgtgccgggcgtgggtgttccgggcgtgggtgttccgggtggcggtgtgccgggcgcaggtgttcctggtgtaggtgtgccgggtgttggtgtgccgggtgttggtgtaccaggtggcggtgttccgggtgcaggcgttccgggtggcggtgtgccgggcgtgggtgttccgggcgtgggtgttccgggtggcggtgtgccgggcgcaggtgttcctggtgtaggtgtgccgggtgttggtgtgccgggtgttggtgtaccaggtggcggtgttccgggtgcaggcgttccgggtggcggtgtgccgggcgtgggtgttccgggcgtgggtgttccgggtggcggtgtgccgggcgcaggtgttcctggtgtaggtgtgccgggtgttggtgtgccgggtgttggtgtaccaggtggcggtgttccgggtgcaggcgttccgggtggcggtgtgccgggcgtgggtgttccgggcgtgggtgttccgggtggcggtgtgccgggcgcaggtgttcctggtgtaggtgtgccgggtgttggtgtgccgggtgttggtgtaccaggtggcggtgttccgggtgcaggcgttccgggtggcggtgtgccgggctggccgtgataagctagcatgactggtggacagcaaatg

SEQ ID NO: 56 - protein, 643 aa, Artificial Sequence
  GLP-1(A8G,7-37)ELP1-120 amino acid sequence
MENLYFQHGEGTFTSDVSSYLEGQAAKEFIAWLVKGRGVPGVGVPGVGVPGGGVPGAGVPGVGVPGVGVPGVGVPGGGVPGAGVPGGGVPGVGVPGVGVPGGGVPGAGVPGVGVPGVGVPGVGVPGGGVPGAGVPGGGVPGVGVPGVGVPGGGVPGAGVPGVGVPGVGVPGVGVPGGGVPGAGVPGGGVPGVGVPGVGVPGGGVPGAGVPGVGVPGVGVPGVGVPGGGVPGAGVPGGGVPGVGVPGVGVPGGGVPGAGVPGVGVPGVGVPGVGVPGGGVPGAGVPGGGVPGVGVPGVGVPGGGVPGAGVPGVGVPGVGVPGVGVPGGGVPGAGVPGGGVPGVGVPGVGVPGGGVPGAGVPGVGVPGVGVPGVGVPGGGVPGAGVPGGGVPGVGVPGVGVPGGGVPGAGVPGVGVPGVGVPGVGVPGGGVPGAGVPGGGVPGVGVPGVGVPGGGVPGAGVPGVGVPGVGVPGVGVPGGGVPGAGVPGGGVPGVGVPGVGVPGGGVPGAGVPGVGVPGVGVPGVGVPGGGVPGAGVPGGGVPGVGVPGVGVPGGGVPGAGVPGVGVPGVGVPGVGVPGGGVPGAGVPGGGVPGVGVPGVGVPGGGVPGAGVPGVGVPGVGVPGVGVPGGGVPGAGVPGGGVPGWP

SEQ ID NO: 57 - DNA, 3700 bp, Artificial Sequence
  pPB0788 DNA sequence
gacggatcgggagatctcccgatcccctatggtgcactctcagtacaatctgctctgatgccgcatagttaagccagtatctgctccctgcttgtgtgttggaggtcgctgagtagtgcgcgagcaaaatttaagctacaacaaggcaaggcttgaccgacaattgcatgaagaatctgcttagggttaggcgttttgcgctgcttcgcgatgtacgggccagatatacgcgttgacattgattattgactagttattaatagtaatcaattacggggtcattagttcatagcccatatatggagttccgcgttacataacttacggtaaatggcccgcctggctgaccgcccaacgacccccgcccattgacgtcaataatgacgtatgttcccatagtaacgccaatagggactttccattgacgtcaatgggtggagtatttacggtaaactgcccacttggcagtacatcaagtgtatcatatgccaagtacgccccctattgacgtcaatgacggtaaatggcccgcctggcattatgcccagtacatgaccttatgggactttcctacttggcagtacatctacgtattagtcatcgctattaccatggtgatgcggttttggcagtacatcaatgggcgtggatagcggtttgactcacggggatttccaagtctccaccccattgacgtcaatgggagtttgttttggcaccaaaatcaacgggactttccaaaatgtcgtaacaactccgccccattgacgcaaatgggcggtaggcgtgtacggtgggaggtctatataagcagagctctctggctaactagagaacccactgcttactggcttatcgaaattaatacgactcactatagggagacccaagctggctagcatggtctcccaggccctcaggctcctctgccttctgcttgggcttcagggctgcctggctgcagtcttcgtaacccaggaggaagcccacggcgtcctgcaccggcgccggcgcgccaacgcgttcctggaggagctacggccgggctccctggagagggagtgcaaggaggagcagtgctccttcgaggaggcccgggagatcttcaaggacgcggagaggacgaagctgttctggatttcttacagtgatggggaccagtgtgcctcaagtccatgccagaatgggggctcctgcaaggaccagctccagtcctatatctgcttctgcctccctgccttcgagggccggaactgtgagacgcacaaggatgaccagctgatctgtgtgaacgagaacggcggctgtgagcagtactgcagtgaccacacgggcaccaagcgctcctgtcggtgccacgaggggtactctctgctggcagacggggtgtcctgcacacccacagttgaatatccatgtggaaaaatacctattctagaaaaaagaaatgccagcaaaccccaaggccgaattgtggggggcaaggtgtgccccaaaggggagtgtccatggcaggtcctgttgttggtgaatggagctcagttgtgtggggggaccctgatcaacaccatctgggtggtctccgcggcccactgtttcgacaaaatcaagaactggaggaacctgatcgcggtgctgggcgagcacgacctcagcgagcacgacggggatgagcagagccggcgggtggcgcaggtcatcatccccagcacgtacgtcccgggcaccaccaaccacgacatcgcgctgctccgcctgcaccagcccgtggtcctcactgaccatgtggtgcccctctgcctgcccgaacggacgttctctgagaggacgctggccttcgtgcgcttctcattggtcagcggctggggccagctgctggaccgtggcgccacggccctggagctcatggtcctcaacgtgccccggctgatgacccaggactgcctgcagcagtcacggaaggtgggagactccccaaatatcacggagtacatgttctgtgccggctactcggatggcagcaaggactcctgcaagggggacagtggaggcccacatgccacccactaccggggcacgtggtacctgacgggcatcgtcagctggggccagggctgcgcaaccgtgggccactttggggtgtacaccagggtctcccagtacatcgagtggctgcaaaagctcatgcgctcagagccacgcccaggagtcctcctgcgagccccatttcccgcggccgctgaaaacctgtattttcagggtggggccgctgggccgggcgtgggagttcccggcgtgggagttcccggaggcggagtgcccggcgcaggagttcctggagtcggagtgcccggagttggagtgcccggagttggagtcccaggaggcggagtccccggagcaggcgtccccggaggcggagtgccgggcgtgggagttcccggcgtgggagttcccggaggcggagtgcccggcgcaggagttcctggagtcggagtgcccggagttggagtgcccggagttggagtcccaggaggcggagtccccggagcaggcgtccccggaggcggagtgccgggcgtgggagttcccggcgtgggagttcccggaggcggagtgcccggcgcaggagttcctggagtcggagtgcccggagttggagtgcccggagttggagtcccaggaggcggagtccccggagcaggcgtccccggaggcggagtgccgggcgtgggagttcccggcgtgggagttcccggaggcggagtgcccggcgcaggagttcctggagtcggagtgcccggagttggagtgcccggagttggagtcccaggaggcggagtccccggagcaggcgtccccggaggcggagtgccgggcgtgggagttcccggcgtgggagttcccggaggcggagtgcccggcgcaggagttcctggagtcggagtgcccggagttggagtgcccggagttggagtcccaggaggcggagtccccggagcaggcgtccccggaggcggagtgccgggcgtgggagttcccggcgtgggagttcccggaggcggagtgcccggcgcaggagttcctggagtcggagtgcccggagttggagtgcccggagttggagtcccaggaggcggagtccccggagcaggcgtccccggaggcggagtgccgggcgtgggagttcccggcgtgggagttcccggaggcggagtgcccggcgcaggagttcctggagtcggagtgcccggagttggagtgcccggagttggagtcccaggaggcggagtccccggagcaggcgtccccggaggcggagtgccgggcgtgggagttcccggcgtgggagttcccggaggcggagtgcccggcgcaggagttcctggagtcggagtgcccggagttggagtgcccggagttggagtcccaggaggcggagtccccggagcaggcgtccccggaggcggagtgccgggcgtgggagttcccggcgtgggagttcccggaggcggagtgcccggcgcaggagttcctggagtcggagtgcccggagttggagtgcccggagttggagtcccaggaggcggagtccccggagcaggcgtccccggaggcggagtgccgggctggccttgatgactcgagtctagagggcccgtttaaacccgctgatcagcctcgactgtgccttctagtt

SEQ ID NO: 58 - protein, 912 aa, Artificial Sequence
  Factor VII-ELP 1-90 amino acid sequence
MVSQALRLLCLLLGLQGCLAAVFVTQEEAHGVLHRRRRANAFLEELRPGSLERECKEEQCSFEEAREIFKDAERTKLFWISYSDGDQCASSPCQNGGSCKDQLQSYICFCLPAFEGRNCETHKDDQLICVNENGGCEQYCSDHTGTKRSCRCHEGYSLLADGVSCTPTVEYPCGKIPILEKRNASKPQGRIVGGKVCPKGECPWQVLLLVNGAQLCGGTLINTIWVVSAAHCFDKIKNWRNLIAVLGEHDLSEHDGDEQSRRVAQVIIPSTYVPGTTNHDIALLRLHQPVVLTDHVVPLCLPERTFSERTLAFVRFSLVSGWGQLLDRGATALELMVLNVPRLMTQDCLQQSRKVGDSPNITEYMFCAGYSDGSKDSCKGDSGGPHATHYRGTWYLTGIVSWGQGCATVGHFGVYTRVSQYIEWLQKLMRSEPRPGVLLRAPFPAAAENLYFQGGAAGPGVGVPGVGVPGGGVPGAGVPGVGVPGVGVPGVGVPGGGVPGAGVPGGGVPGVGVPGVGVPGGGVPGAGVPGVGVPGVGVPGVGVPGGGVPGAGVPGGGVPGVGVPGVGVPGGGVPGAGVPGVGVPGVGVPGVGVPGGGVPGAGVPGGGVPGVGVPGVGVPGGGVPGAGVPGVGVPGVGVPGVGVPGGGVPGAGVPGGGVPGVGVPGVGVPGGGVPGAGVPGVGVPGVGVPGVGVPGGGVPGAGVPGGGVPGVGVPGVGVPGGGVPGAGVPGVGVPGVGVPGVGVPGGGVPGAGVPGGGVPGVGVPGVGVPGGGVPGAGVPGVGVPGVGVPGVGVPGGGVPGAGVPGGGVPGVGVPGVGVPGGGVPGAGVPGVGVPGVGVPGVGVPGGGVPGAGVPGGGVPGVGVPGVGVPGGGVPGAGVPGVGVPGVGVPGVGVPGGGVPGAGVPGGGVPGWP

SEQ ID NO: 59 - protein, 31 aa, Unknown
  GLP-1 receptor agonist
HGEGTFTSDVSSYLEGQAAKEFIAWLVKGRG